European Patent Application EP 3 858 865 A9, published February 14, 2024. Title: FUSION PROTEIN OF MUTATED SINGLE-CHAIN HUMAN COAGULATION FACTOR VIII, PREPARATION METHOD THEREFOR, AND USE THEREOF. Applicant: AMPSOURCE BIOPHARMA SHANGHAI INC. PHARMAB, INC. The sequence listing filed with the application follows.

SEQUENCE LISTING (11 sequences)

SEQ ID NO: 1 - protein, 2351 aa, Full-length FVIII amino acid sequence
MQIELSTCFFLCLLRFCFSATRRYYLGAVELSWDYMQSDLGELPVDARFPPRVPKSFPFNTSVVYKKTLFVEFTDHLFNIAKPRPPWMGLLGPTIQAEVYDTVVITLKNMASHPVSLHAVGVSYWKASEGAEYDDQTSQREKEDDKVFPGGSHTYVWQVLKENGPMASDPLCLTYSYLSHVDLVKDLNSGLIGALLVCREGSLAKEKTQTLHKFILLFAVFDEGKSWHSETKNSLMQDRDAASARAWPKMHTVNGYVNRSLPGLIGCHRKSVYWHVIGMGTTPEVHSIFLEGHTFLVRNHRQASLEISPITFLTAQTLLMDLGQFLLFCHISSHQHDGMEAYVKVDSCPEEPQLRMKNNEEAEDYDDDLTDSEMDVVRFDDDNSPSFIQIRSVAKKHPKTWVHYIAAEEEDWDYAPLVLAPDDRSYKSQYLNNGPQRIGRKYKKVRFMAYTDETFKTREAIQHESGILGPLLYGEVGDTLLIIFKNQASRPYNIYPHGITDVRPLYSRRLPKGVKHLKDFPILPGEIFKYKWTVTVEDGPTKSDPRCLTRYYSSFVNMERDLASGLIGPLLICYKESVDQRGNQIMSDKRNVILFSVFDENRSWYLTENIQRFLPNPAGVQLEDPEFQASNIMHSINGYVFDSLQLSVCLHEVAYWYILSIGAQTDFLSVFFSGYTFKHKMVYEDTLTLFPFSGETVFMSMENPGLWILGCHNSDFRNRGMTALLKVSSCDKNTGDYYEDSYEDISAYLLSKNNAIEPRSFSQNSRHPSTRQKQFNATTIPENDIEKTDPWFAHRTPMPKIQNVSSSDLLMLLRQSPTPHGLSLSDLQEAKYETFSDDPSPGAIDSNNSLSEMTHFRPQLHHSGDMVFTPESGLQLRLNEKLGTTAATELKKLDFKVSSTSNNLISTIPSDNLAAGTDNTSSLGPPSMPVHYDSQLDTTLFGKKSSPLTESGGPLSLSEENNDSKLLESGLMNSQESSWGKNVSSTESGRLFKGKRAHGPALLTKDNALFKVSISLLKTNKTSNNSATNRKTHIDGPSLLIENSPSVWQNILESDTEFKKVTPLIHDRMLMDKNATALRLNHMSNKTTSSKNMEMVQQKKEGPIPPDAQNPDMSFFKMLFLPESARWIQRTHGKNSLNSGQGPSPKQLVSLGPEKSVEGQNFLSEKNKVVVGKGEFTKDVGLKEMVFPSSRNLFLTNLDNLHENNTHNQEKKIQEEIEKKETLIQENVVLPQIHTVTGTKNFMKNLFLLSTRQNVEGSYDGAYAPVLQDFRSLNDSTNRTKKHTAHFSKKGEEENLEGLGNQTKQIVEKYACTTRISPNTSQQNFVTQRSKRALKQFRLPLEETELEKRIIVDDTSTQWSKNMKHLTPSTLTQIDYNEKEKGAITQSPLSDCLTRSHSIPQANRSPLPIAKVSSFPSIRPIYLTRVLFQDNSSHLPAASYRKKDSGVQESSHFLQGAKKNNLSLAILTLEMTGDQREVGSLGTSATNSVTYKKVENTVLPKPDLPKTSGKVELLPKVHIYQKDLFPTETSNGSPGHLDLVEGSLLQGTEGAIKWNEANRPGKVPFLRVATESSAKTPSKLLDPLAWDNHYGTQIPKEEWKSQEKSPEKTAFKKKDTILSLNACESNHAIAAINEGQNKPEIEVTWAKQGRTERLCSQNPPVLKRHQREITRTTLQSDQEEIDYDDTISVEMKKEDFDIYDEDENQSPRSFQKKTRHYFIAAVERLWDYGMSSSPHVLRNRAQSGSVPQFKKVVFQEFTDGSFTQPLYRGELNEHLGLLGPYIRAEVEDNIMVTFRNQASRPYSFYSSLISYEEDQRQGAEPRKNFVKPNETKTYFWKVQHHMAPTKDEFDCKAWAYFSDVDLEKDVHSGLIGPLLVCHTNTLNPAHGRQVTVQEFALFFTIFDETKSWYFTENMERNCRAPCNIQMEDPTFKENYRFHAINGYIMDTLPGLVMAQDQRIRWYLLSMGSNENIHSIHFSGHVFTVRKKEEYKMALYNLYPGVFETVEMLPSKAGIWRVECLIGEHLHAGMSTLFLVYSNKCQTPLGMASGHIRDFQITASGQYGQWAPKLARLHYSGSINAWSTKEPFSWIKVDLLAPMIIHGIKTQGARQKFSSLYISQFIIMYSLDGKKWQTYRGNSTGTLMVFFGNVDSSGIKHNIFNPPIIARYIRLHPTHYSIRSTLRMELMGCDLNSCSMPLGMESKAISDAQITASSYFTNMFATWSPSKARLHLQGRSNAWRPQVNNPKEWLQVDFQKTMKVTGVTTQGVKSLLTSMYVKEFLISSSQDGHQWTLFFQNGKVKVFQGNQDSFTPVVNSLDPPLLTRYLRIHPQSWVHQIALRMEVLGCEAQDLY

SEQ ID NO: 2 - protein, 1445 aa, scFVIII amino acid sequence
ATRRYYLGAVELSWDYMQSDLGELPVDARFPPRVPKSFPFNTSVVYKKTLFVEFTDHLFNIAKPRPPWMGLLGPTIQAEVYDTVVITLKNMASHPVSLHAVGVSYWKASEGAEYDDQTSQREKEDDKVFPGGSHTYVWQVLKENGPMASDPLCLTYSYLSHVDLVKDLNSGLIGALLVCREGSLAKEKTQTLHKFILLFAVFDEGKSWHSETKNSLMQDRDAASARAWPKMHTVNGYVNRSLPGLIGCHRKSVYWHVIGMGTTPEVHSIFLEGHTFLVRNHRQASLEISPITFLTAQTLLMDLGQFLLFCHISSHQHDGMEAYVKVDSCPEEPQLRMKNNEEAEDYDDDLTDSEMDVVRFDDDNSPSFIQIRSVAKKHPKTWVHYIAAEEEDWDYAPLVLAPDDRSYKSQYLNNGPQRIGRKYKKVRFMAYTDETFKTREAIQHESGILGPLLYGEVGDTLLIIFKNQASRPYNIYPHGITDVRPLYSRRLPKGVKHLKDFPILPGEIFKYKWTVTVEDGPTKSDPRCLTRYYSSFVNMERDLASGLIGPLLICYKESVDQRGNQIMSDKRNVILFSVFDENRSWYLTENIQRFLPNPAGVQLEDPEFQASNIMHSINGYVFDSLQLSVCLHEVAYWYILSIGAQTDFLSVFFSGYTFKHKMVYEDTLTLFPFSGETVFMSMENPGLWILGCHNSDFRNRGMTALLKVSSCDKNTGDYYEDSYEDISAYLLSKNNAIEPRSFSQNSRHPSTRQKQFNATTIPENRTTLQSDQEEIDYDDTISVEMKKEDFDIYDEDENQSPRSFQKKTRHYFIAAVERLWDYGMSSSPHVLRNRAQSGSVPQFKKVVFQEFTDGSFTQPLYRGELNEHLGLLGPYIRAEVEDNIMVTFRNQASRPYSFYSSLISYEEDQRQGAEPRKNFVKPNETKTYFWKVQHHMAPTKDEFDCKAWAYFSDVDLEKDVHSGLIGPLLVCHTNTLNPAHGRQVTVQEFALFFTIFDETKSWYFTENMERNCRAPCNIQMEDPTFKENYRFHAINGYIMDTLPGLVMAQDQRIRWYLLSMGSNENIHSIHFSGHVFTVRKKEEYKMALYNLYPGVFETVEMLPSKAGIWRVECLIGEHLHAGMSTLFLVYSNKCQTPLGMASGHIRDFQITASGQYGQWAPKLARLHYSGSINAWSTKEPFSWIKVDLLAPMIIHGIKTQGARQKFSSLYISQFIIMYSLDGKKWQTYRGNSTGTLMVFFGNVDSSGIKHNIFNPPIIARYIRLHPTHYSIRSTLRMELMGCDLNSCSMPLGMESKAISDAQITASSYFTNMFATWSPSKARLHLQGRSNAWRPQVNNPKEWLQVDFQKTMKVTGVTTQGVKSLLTSMYVKEFLISSSQDGHQWTLFFQNGKVKVFQGNQDSFTPVVNSLDPPLLTRYLRIHPQSWVHQIALRMEVLGCEAQDLY

SEQ ID NO: 3 - protein, 33 aa, hCGbeta CTP full-length amino acid sequence
PRFQDSSSSKAPPPSLPSPSRLPGPSDTPILPQ

SEQ ID NO: 4 - protein, 227 aa, vFcgamma1 amino acid sequence
DKTHTCPPCPAPEVAGGPSVFLFPPKPKDTLMISRTPEVTCVVVDVSHEDPEVKFNWYVDGVEVHNAKTKPREEQYNSTYRVVSVLTVLHQDWLNGKEYKCKVSNKALPASIEKTISKAKGQPREPQVYTLPPSRDELTKNQVSLTCLVKGFYPSDIAVEWESNGQPENNYKTTPPVLDSDGSFFLYSKLTVDKSRWQQGNVFSCSVMHEALHNHYTQKSLSLSPGK

SEQ ID NO: 5 - protein, 223 aa, vFcgamma2-1 amino acid sequence
VECPPCPAPPVAGPSVFLFPPKPKDTLMISRTPEVTCVVVDVSHEDPEVQFNWYVDGVEVHNAKTKPREEQFNSTFRVVSVLTVVHQDWLNGKEYKCKVSNKGLPASIEKTISKTKGQPREPQVYTLPPSREEMTKNQVSLTCLVKGFYPSDIAVEWESNGQPENNYKTTPPMLDSDGSFFLYSKLTVDKSRWQQGNVFSCSVMHEALHNHYTQKSLSLSPGK

SEQ ID NO: 6 - protein, 223 aa, vFcgamma2-2 amino acid sequence
VECPPCPAPPVAGPSVFLFPPKPKDQLMISRTPEVTCVVVDVSHEDPEVQFNWYVDGVEVHNAKTKPREEQFNSTFRVVSVLTVVHQDWLNGKEYKCKVSNKGLPAPIEKTISKTKGQPREPQVYTLPPSREEMTKNQVSLTCLVKGFYPSDIAVEWESNGQPENNYKTTPPMLDSDGSFFLYSKLTVDKSRWQQGNVFSCSVLHEALHNHYTQKSLSLSPGK

SEQ ID NO: 7 - protein, 223 aa, vFcgamma2-3 amino acid sequence
VECPPCPAPPVAGPSVFLFPPKPKDQLMISRTPEVTCVVVDVSHEDPEVQFNWYVDGVEVHNAKTKPREEQFNSTFRVVSVLTVVHQDWLNGKEYKCKVSNKGLPASIEKTISKTKGQPREPQVYTLPPSREEMTKNQVSLTCLVKGFYPSDIAVEWESNGQPENNYKTTPPMLDSDGSFFLYSKLTVDKSRWQQGNVFSCSVLHEALHNHYTQKSLSLSPGK

SEQ ID NO: 8 - protein, 229 aa, vFcgamma4 amino acid sequence
ESKYGPPCPPCPAPEFAGGPSVFLFPPKPKDTLMISRTPEVTCVVVDVSQEDPEVQFNWYVDGVEVHNAKTKPREEQFNSTYRVVSVLTVLHQDWLNGKEYKCKVSNKGLPSSIEKTISKAKGQPREPQVYTLPPSQEEMTKNQVSLTCLVKGFYPSDIAVEWESNGQPENNYKTTPPVLDSDGSFFLYSRLTVDKSRWQEGNVFSCSVMHEALHNHYTQKSLSLSLGK

SEQ ID NO: 9 - protein, 1723 aa, amino acid sequence of scFVIII fusion protein
ATRRYYLGAVELSWDYMQSDLGELPVDARFPPRVPKSFPFNTSVVYKKTLFVEFTDHLFNIAKPRPPWMGLLGPTIQAEVYDTVVITLKNMASHPVSLHAVGVSYWKASEGAEYDDQTSQREKEDDKVFPGGSHTYVWQVLKENGPMASDPLCLTYSYLSHVDLVKDLNSGLIGALLVCREGSLAKEKTQTLHKFILLFAVFDEGKSWHSETKNSLMQDRDAASARAWPKMHTVNGYVNRSLPGLIGCHRKSVYWHVIGMGTTPEVHSIFLEGHTFLVRNHRQASLEISPITFLTAQTLLMDLGQFLLFCHISSHQHDGMEAYVKVDSCPEEPQLRMKNNEEAEDYDDDLTDSEMDVVRFDDDNSPSFIQIRSVAKKHPKTWVHYIAAEEEDWDYAPLVLAPDDRSYKSQYLNNGPQRIGRKYKKVRFMAYTDETFKTREAIQHESGILGPLLYGEVGDTLLIIFKNQASRPYNIYPHGITDVRPLYSRRLPKGVKHLKDFPILPGEIFKYKWTVTVEDGPTKSDPRCLTRYYSSFVNMERDLASGLIGPLLICYKESVDQRGNQIMSDKRNVILFSVFDENRSWYLTENIQRFLPNPAGVQLEDPEFQASNIMHSINGYVFDSLQLSVCLHEVAYWYILSIGAQTDFLSVFFSGYTFKHKMVYEDTLTLFPFSGETVFMSMENPGLWILGCHNSDFRNRGMTALLKVSSCDKNTGDYYEDSYEDISAYLLSKNNAIEPRSFSQNSRHPSTRQKQFNATTIPENRTTLQSDQEEIDYDDTISVEMKKEDFDIYDEDENQSPRSFQKKTRHYFIAAVERLWDYGMSSSPHVLRNRAQSGSVPQFKKVVFQEFTDGSFTQPLYRGELNEHLGLLGPYIRAEVEDNIMVTFRNQASRPYSFYSSLISYEEDQRQGAEPRKNFVKPNETKTYFWKVQHHMAPTKDEFDCKAWAYFSDVDLEKDVHSGLIGPLLVCHTNTLNPAHGRQVTVQEFALFFTIFDETKSWYFTENMERNCRAPCNIQMEDPTFKENYRFHAINGYIMDTLPGLVMAQDQRIRWYLLSMGSNENIHSIHFSGHVFTVRKKEEYKMALYNLYPGVFETVEMLPSKAGIWRVECLIGEHLHAGMSTLFLVYSNKCQTPLGMASGHIRDFQITASGQYGQWAPKLARLHYSGSINAWSTKEPFSWIKVDLLAPMIIHGIKTQGARQKFSSLYISQFIIMYSLDGKKWQTYRGNSTGTLMVFFGNVDSSGIKHNIFNPPIIARYIRLHPTHYSIRSTLRMELMGCDLNSCSMPLGMESKAISDAQITASSYFTNMFATWSPSKARLHLQGRSNAWRPQVNNPKEWLQVDFQKTMKVTGVTTQGVKSLLTSMYVKEFLISSSQDGHQWTLFFQNGKVKVFQGNQDSFTPVVNSLDPPLLTRYLRIHPQSWVHQIALRMEVLGCEAQDLYGSGGGGSGGGGSGGGGSGGGGSGGGGSSSSSKAPPPSLPSPSRLPGPSDTPILPQVECPPCPAPPVAGPSVFLFPPKPKDQLMISRTPEVTCVVVDVSHEDPEVQFNWYVDGVEVHNAKTKPREEQFNSTFRVVSVLTVVHQDWLNGKEYKCKVSNKGLPASIEKTISKTKGQPREPQVYTLPPSREEMTKNQVSLTCLVKGFYPSDIAVEWESNGQPENNYKTTPPMLDSDGSFFLYSKLTVDKSRWQQGNVFSCSVLHEALHNHYTQKSLSLSPGK

SEQ ID NO: 10 - DNA, 5169 bp, nucleotide sequence of scFVIII fusion protein
gccaccaggaggtactacctcggagccgtcgagctcagctgggattatatgcagagcgacctcggagaactccctgtcgatgccaggtttcccccccgggtgcccaagtccttcccctttaacacctccgtcgtctacaagaagaccctgttcgtcgagttcacagaccatctgttcaatattgctaaacccaggcccccctggatgggactgctgggccccacaatccaagccgaggtgtatgataccgtggtgatcaccctcaagaatatggcttcccatcccgtctccctgcacgccgtcggcgtgtcctactggaaggcctccgaaggcgccgagtacgatgatcagacaagccagcgggagaaggaggatgataaggtctttcccggaggttctcacacctatgtctggcaggtgctgaaagagaacggccccatggctagcgaccccctgtgcctcacctattcctacctcagccatgtggacctggtgaaggatctgaactccggcctgattggcgccctcctggtctgcagggagggaagcctggccaaagaaaagacccagaccctgcataaattcatcctcctgtttgccgtcttcgatgagggcaagtcctggcactccgaaacaaagaactccctgatgcaggacagggacgctgcctccgccagggcctggcccaagatgcacaccgtcaacggatacgtgaataggtccctccccggcctgattggatgccatcggaagtccgtgtattggcacgtgatcggcatgggaaccacacccgaagtgcactccatcttcctggaaggacatacatttctcgtccggaaccaccggcaggcttccctggaaatctcccctatcaccttcctgaccgctcagacactgctgatggatctgggccagttcctgctgttctgccacatttcctcccaccagcacgacggcatggaggcttatgtcaaggtggatagctgccccgaggaaccccagctgcggatgaaaaacaatgaggaagccgaggactacgacgatgacctcaccgatagcgagatggacgtggtcaggttcgacgacgataactccccttccttcatccagatccggagcgtggccaagaagcaccccaaaacctgggtgcactacatcgccgctgaggaggaagactgggactatgctcctctcgtgctggcccccgatgacaggtcctacaaaagccagtatctgaacaatggaccccagcggattggaaggaagtataagaaagtccggtttatggcttacaccgacgagacctttaaaacccgggaagccatccagcacgagagcggcatcctcggccctctcctgtacggagaggtcggagacacactcctcatcatttttaagaaccaggcctcccggccctacaacatctatcctcatggcatcaccgatgtgaggcctctgtacagcaggaggctgcccaaaggagtcaagcacctgaaagatttccctatcctccccggagagatcttcaagtacaaatggaccgtcaccgtggaggacggccccacaaagtccgatccccggtgcctgacccggtactattccagctttgtcaacatggagcgggacctcgccagcggcctgatcggccctctgctcatctgctataaggagtccgtcgatcagaggggaaaccagatcatgtccgataagcggaatgtgatcctgttttccgtgtttgacgaaaaccggtcctggtatctgaccgagaacatccagcggtttctgcctaaccccgctggcgtgcaactggaagatcctgagttccaggcttccaatatcatgcacagcatcaacggctacgtcttcgacagcctgcagctgtccgtctgcctgcacgaagtcgcctactggtacattctcagcattggcgcccagacagacttcctgtccgtctttttctccggctataccttcaaacataagatggtctacgaggataccctcacactgttccctttcagcggcgaaaccgtgtttatgagcatggaaaatcccggcctgtggattttaggatgccacaactccgatttcaggaataggggcatgacagctctcctcaaagtgtcctcctgcgacaagaacacaggcgactactacgaggacagctatgaggatatttccgcctacctgctcagcaagaataatgccatcgagcctaggtccttctcccaaaactcccggcatcccagcacccggcagaagcagttcaatgccaccacaattcctgaaaatagaacaaccctgcagtccgaccaggaggaaatcgactacgatgacaccatctccgtcgagatgaagaaggaagacttcgacatctatgacgaggacgaaaaccagagccctcggtcctttcagaaaaaaacacggcattactttatcgctgccgtcgaacggctgtgggactacggcatgagctcctccccccatgtgctccggaatcgggctcaatccggctccgtgcctcagtttaagaaggtggtgtttcaagagttcaccgacggcagctttacacagcccctgtacaggggagagctgaacgagcacctgggactgctcggaccttacattcgggccgaagtcgaggataacatcatggtgacctttaggaatcaggcttcccggccttactccttctactccagcctcatctcctacgaagaagaccaacggcagggcgccgagcctcggaagaatttcgtgaagcccaatgaaaccaaaacatacttttggaaagtccagcaccacatggcccctaccaaggatgagttcgactgcaaagcctgggcctatttctccgatgtggatctggagaaggacgtccattccggactgatcggccccctcctcgtctgccacaccaacaccctcaatcctgcccacggcaggcaggtgacagtccaggagttcgccctgtttttcaccatctttgacgagaccaagtcctggtactttaccgagaatatggaaaggaattgcagggccccctgcaacattcagatggaggaccccaccttcaaagagaactaccggtttcatgccattaatggatacatcatggacacactgcccggcctggtgatggctcaggaccaacggattcggtggtacctgctgagcatgggctccaacgaaaatatccacagcatccactttagcggccacgtgtttaccgtgcggaagaaggaggagtataaaatggccctctacaacctctatcccggcgtgttcgaaacagtcgagatgctccctagcaaggccggaatctggagggtggaatgcctgattggcgaacatctgcacgccggaatgagcaccctcttcctggtctacagcaacaaatgtcagacccctctgggcatggcttccggccacatcagggactttcagattaccgctagcggacaatatggccagtgggcccctaaactcgctaggctgcactacagcggaagcatcaacgcctggtccacaaaggaacctttctcctggatcaaggtggatctcctcgcccctatgatcatccatggcatcaagacccaaggcgctaggcagaagtttagctccctgtacatcagccagtttatcatcatgtactccctcgacggcaagaagtggcagacataccggggaaactccacaggcaccctgatggtgttctttggcaacgtggacagcagcggaattaagcataatattttcaaccctcctatcatcgccaggtacatccggctgcaccctacacactacagcatcaggagcaccctgaggatggagctgatgggctgcgatctgaatagctgctccatgcccctcggcatggagagcaaggctatttccgacgcccaaattaccgccagctcctatttcaccaacatgttcgccacatggagccctagcaaagctcggctccatctccagggcaggtccaacgcctggcggcctcaggtgaataatcccaaagaatggctgcaggtcgacttccagaagacaatgaaagtgaccggcgtgaccacccagggagtcaaaagcctcctcaccagcatgtacgtcaaagagttcctgatcagctcctcccaggacggacatcaatggacactcttttttcagaacggcaaggtgaaggtgttccagggcaaccaggattcctttacccctgtggtcaactccttagatcctcccctcctgacacggtacctgcggattcaccctcagtcctgggtgcatcagatcgctctgaggatggaagtgctcggctgcgaagcccaagacctgtacggatccggtggcggtggctccggtggaggcggaagcggcggtggaggatcaggcggtggaggtagcggcggaggcggtagctccagctctagtaaagctccccctccttccctgccctcaccctcaagactgcctggaccttccgacactcccatcctgccacaggtggagtgccctccatgtccagcaccccctgtcgcaggtccatctgtgttcctgtttccacccaagcctaaagaccagctgatgatctcccgcaccccagaagtcacctgtgtggtcgtggatgtgagccatgaagaccccgaggtccagttcaattggtacgtggatggcgtcgaggtgcacaacgctaagacaaaacctagagaagagcagttcaactctacctttcgcgtcgtgagtgtgctgacagtcgtgcaccaggactggctgaatggcaaggagtataagtgcaaagtgagcaacaaaggactgcctgcctcaatcgaaaagactatttccaagaccaaaggacagccaagagagccccaggtgtacaccctgcctccaagccgcgaagagatgactaaaaatcaggtctctctgacctgtctggtgaaggggttttatcctagtgatatcgccgtggaatgggagtcaaacggtcagccagagaacaattacaagaccacaccccctatgctggacagcgatgggtctttctttctgtatagcaaactgacagtggacaagtctcggtggcagcagggtaacgtcttctcttgcagtgtgctgcacgaagcactgcacaatcattacacccagaagtcactgtcactgagcccaggaaaa

SEQ ID NO: 11 - protein, 1716 aa, amino acid sequence of DS-F8 fusion protein
ATRRYYLGAVELSWDYMQSDLGELPVDARFPPRVPKSFPFNTSVVYKKTLFVEFTDHLFNIAKPRPPWMGLLGPTIQAEVYDTVVITLKNMASHPVSLHAVGVSYWKASEGAEYDDQTSQREKEDDKVFPGGSHTYVWQVLKENGPMASDPLCLTYSYLSHVDLVKDLNSGLIGALLVCREGSLAKEKTQTLHKFILLFAVFDEGKSWHSETKNSLMQDRDAASARAWPKMHTVNGYVNRSLPGLIGCHRKSVYWHVIGMGTTPEVHSIFLEGHTFLVRNHRQASLEISPITFLTAQTLLMDLGQFLLFCHISSHQHDGMEAYVKVDSCPEEPQLRMKNNEEAEDYDDDLTDSEMDVVRFDDDNSPSFIQIRSVAKKHPKTWVHYIAAEEEDWDYAPLVLAPDDRSYKSQYLNNGPQRIGRKYKKVRFMAYTDETFKTREAIQHESGILGPLLYGEVGDTLLIIFKNQASRPYNIYPHGITDVRPLYSRRLPKGVKHLKDFPILPGEIFKYKWTVTVEDGPTKSDPRCLTRYYSSFVNMERDLASGLIGPLLICYKESVDQRGNQIMSDKRNVILFSVFDENRSWYLTENIQRFLPNPAGVQLEDPEFQASNIMHSINGYVFDSLQLSVCLHEVAYWYILSIGAQTDFLSVFFSGYTFKHKMVYEDTLTLFPFSGETVFMSMENPGLWILGCHNSDFRNRGMTALLKVSSCDKNTGDYYEDSYEDISAYLLSKNNAIEPRSFSQNPPVLKRHQREITRTTLQSDQEEIDYDDTISVEMKKEDFDIYDEDENQSPRSFQKKTRHYFIAAVERLWDYGMSSSPHVLRNRAQSGSVPQFKKVVFQEFTDGSFTQPLYRGELNEHLGLLGPYIRAEVEDNIMVTFRNQASRPYSFYSSLISYEEDQRQGAEPRKNFVKPNETKTYFWKVQHHMAPTKDEFDCKAWAYFSDVDLEKDVHSGLIGPLLVCHTNTLNPAHGRQVTVQEFALFFTIFDETKSWYFTENMERNCRAPCNIQMEDPTFKENYRFHAINGYIMDTLPGLVMAQDQRIRWYLLSMGSNENIHSIHFSGHVFTVRKKEEYKMALYNLYPGVFETVEMLPSKAGIWRVECLIGEHLHAGMSTLFLVYSNKCQTPLGMASGHIRDFQITASGQYGQWAPKLARLHYSGSINAWSTKEPFSWIKVDLLAPMIIHGIKTQGARQKFSSLYISQFIIMYSLDGKKWQTYRGNSTGTLMVFFGNVDSSGIKHNIFNPPIIARYIRLHPTHYSIRSTLRMELMGCDLNSCSMPLGMESKAISDAQITASSYFTNMFATWSPSKARLHLQGRSNAWRPQVNNPKEWLQVDFQKTMKVTGVTTQGVKSLLTSMYVKEFLISSSQDGHQWTLFFQNGKVKVFQGNQDSFTPVVNSLDPPLLTRYLRIHPQSWVHQIALRMEVLGCEAQDLYGSGGGGSGGGGSGGGGSGGGGSGGGGSSSSSKAPPPSLPSPSRLPGPSDTPILPQVECPPCPAPPVAGPSVFLFPPKPKDQLMISRTPEVTCVVVDVSHEDPEVQFNWYVDGVEVHNAKTKPREEQFNSTFRVVSVLTVVHQDWLNGKEYKCKVSNKGLPASIEKTISKTKGQPREPQVYTLPPSREEMTKNQVSLTCLVKGFYPSDIAVEWESNGQPENNYKTTPPMLDSDGSFFLYSKLTVDKSRWQQGNVFSCSVLHEALHNHYTQKSLSLSPGK